European Patent Application EP 4 768 912 A1, published July 1, 2026. Title: Methods of immunological assay, reagents for immunological assay, sample pretreatment solutions for immunological assay, and reagent kits for immunological assay, nonspecific reaction inhibitors. Applicant: c/o SEKISUI MEDICAL CO., LTD. The sequence listing filed with the application follows.

SEQUENCE LISTING (1 sequence)

SEQ ID NO: 1 - protein, 452 aa, Homo sapiens
SSGSASAPTLFPLVSCENSNPSSTVAVGCLAQDFLPDSITFSWKYNQSQKISSTRGFPSVLRGGKYAATSQVLLPSKDVMQGTDEHVCKWVQHPNGNKQKNVPLPVIAELPPKVSVFVPPRDGFFGNPRKSKLICQATGFSPRQVWSLREGKQVGSGVTTDQVQAEAKESGPTTYKVTSTLTIKESDWLGESMFTCRVDHRGLTFQQNASSMCVPDQDTAIRVFAIPPSFASIFLTKSTKLTCLVTDLTTYDSVTISWTREENGAVKTHTNISESHPNATFSAVGEASICEDDDWSGERFTCTVTHTDLPSPLKQTISRPKGVALHRPDVYLLPPAREQLNLRESATITCLVTGFSPADVFVQWMQRGEPLSPEKYVTSAPMPEPQAPGRYFAHSILTVSEEEWNTGQTYTCVVAHEALPNRVTERTVDKSTGKPTLYNVSLVMSDTAGTCY